European Patent Application EP 4 212 609 A1, published July 19, 2023. Title: ALPHA-AMYLASE VARIANTS AND POLYNUCLEOTIDES ENCODING SAME. Applicant: Novozymes A/S. The sequence listing filed with the application follows.

SEQUENCE LISTING (17 sequences)

SEQ ID NO: 1 - DNA, 1458 bp, Bacillus sp.
  source 1..1458: mol_type = genomic DNA
catcacgatgggacgaacggaacgattatgcagtattttgaatggaacgttccgaatgatggacaacattggaaccgcttacacaacaacgctcaaaatttaaaaaatgccggaattacagcaatctggattccacctgcgtggaaaggaacgagccaaaatgatgtaggctacggtgcgtatgacctttatgaccttggtgaatttaaccaaaaaggaacggtccgtacgaaatatggaacaaaagcagaattagaacgagcgattcgttcgttaaaggcgaacgggattcaagtgtatggcgatgttgttatgaaccataaaggcggagctgatttcaccgagcgtgttcaagcggttgaagtgaacccgcaaaaccgaaaccaagaagtgtctggcacttatcaaatcgaagcatggacagggttcaattttcctggacgtggcaatcaacattcttcgtttaaatggcgctggtatcatttcgatgggacggattgggaccagtctcgccaactcgcaaatcgtatttataagtttagaggagacggaaaagcatgggactgggaagttgacactgaaaatgggaactatgattacttaatgtatgcagacgttgacatggatcatccagaagtgattaacgaactaaaccgttggggcgtctggtacgcgaatacccttaatttagacggcttccgactggatgcagtgaaacatattaaatttagcttcatgcgtgattggttagggcatgttcgcgggcaaacgggcaagaatctttttgccgttgcagagtattggaagaatgacctaggggctttagaaaattatttaagcaaaacaaattggacgatgagcgcctttgatgttccgcttcattacaacctttatcaagcgtcaaatagtagcggaaattacgacatgagaaacttgttaaatggaacactcgttcaacgtcatccgagccatgcggttacgtttgtcgataaccacgacacacagcctggagaagccctcgaatcgttcgttcaaggctggtttaaaccactagcttatgcaacgattcttacgagagagcaaggctacccacaagtgttttacggcgattattatggcatcccaagtgacggtgttccaagctaccgtcaacagatcgacccacttttaaaagctcgtcaacaatatgcttatggtagacagcacgattactttgatcattgggatgtaattggctggacacgtgaaggaaacgcatctcacccgaactcaggacttgcaaccattatgtctgatggtccaggtggatcaaaatggatgtatgttggccgtcagaaagctggcgaagtgtggcatgacatgactggaaaccgcagtggcactgtgacaattaatcaagacggctggggacacttttttgtcaacggcggctctgtctccgtatgggtgaaacgataa

SEQ ID NO: 2 - DNA, 1539 bp, Alicyclobacillus sp.
  source 1..1539: mol_type = genomic DNA
atgaaaatccgcaacggttggaaaaaaaccttgacgctgttatttgcgctcatcttcttgctgcctcattctgcagccgcgacctttgccggggacaacggcacgatgatgcaatactttgaatggtatctgcccaacgacgggacgctttggaccaagatgggcagcgacgcgtcgcacctgaagtcgatcgggatcaccggcgtctggttcccgccggcgtacaaaggccaatcgcagtcggacgtcggctacggcgtatacgacatgtacgacctcggcgaattcaaccaaaaaggaaccgtccgcaccaagtacggcaccaaagcccagctccaatcggcgatcacctccctgcacaacaacggcatccaagcctacggggacgtcgtcctcaaccaccgcatgggcgccgatgcgacggagacgatctccgccgtggaagtcaacccgtccaaccgcaaccaagtcacctccggggcttacaacatctccgcttggaccgacttcgaattcccgggccgcggcaacacctactcctcgtttaagtggcactcctactactttgacggcgtggactgggaccaatcccgccagctgagcggcaagatctaccagatccaaggcaccggcaaagcgtgggactgggaagtcgattccgaaaacggcaactacgactacctgatgggcgcggacatcgactacgaccacccggacgtgcaaacggaagtgaagaactggggcaagtggttcgtcaacaccctcaacctcgacggcgtgcgcctcgacgcggtcaagcacatcaagttcgactacatgtcttcctggctgtccagcgtcaaatccacgaccggcaagtccaacctgttcgccgtcggcgaatactggaacacctcgctcggagcgctggagaactacgagaacaaaaccaactggagcatgtcgctgttcgacgtgccgctgcacatgaacttccaagcggcagcgaacggcggcggctactatgatatgcgcaacctgctcaacaacacgatgatgaaaaatcacccgatccaagcggtcaccttcgtcgacaaccacgacaccgagccgggccaagccctgcaatcgtgggtatccgactggttcaaaccgctggcctacgcgacgatcctgacccgtcaagaaggctacccgtgcgtgttctacggcgactactacggcatcccgtcgcaaagcgtctccgcgaaatccacctggttggacaagcagctttccgcacgcaaatcctacgcgtacggcacccagcacgactacttggacaaccaagacgtgatcggctggacgcgcgaaggcgattccgcgcacgcgggctcgggtcttgccaccgtcatgtcggacggccctggcggctccaagacgatgtacgtcggcaccgcccatgccggccaagtcttcaaggacatcaccggcaaccgcaccgacaccgtcacgatcaactccgcaggcaacggcaccttcccctgcaacggcggctccgtctcgatctgggtcaaacaa

SEQ ID NO: 3 - DNA, 1560 bp, Bacillus amyloliquefaciens
  source 1..1560: mol_type = genomic DNA
atgagagggagaggaaacatgattcaaaaacgaaagcggacagtttcgttcagacttgtgcttatgtgcacgctgttatttgtcagtttgccgattacaaaaacatcagccgtaaatggcacgctgatgcagtattttgaatggtatacgccgaacgacggccagcattggaaacgattgcagaatgatgcggaacatttatcggatatcggaatcactgccgtctggattcctcccgcatacaaaggattgagccaatccgataacggatacggaccttatgatttgtatgatttaggagaattccagcaaaaagggacggtcagaacgaaatacggcacaaaatcagagcttcaagatgcgatcggctcactgcattcccggaacgtccaagtatacggagatgtggttttgaatcataaggctggtgctgatgcaacagaagatgtaactgccgtcgaagtcaatccggccaatagaaatcaggaaacttcggaggaatatcaaatcaaagcgtggacggattttcgttttccgggccgtggaaacacgtacagtgattttaaatggcattggtatcatttcgacggagcggactgggatgaatcccggaagatcagccgcatctttaagtttcgtggggaaggaaaagcgtgggattgggaagtatcaagtgaaaacggcaactatgactatttaatgtatgctgatgttgactacgaccaccctgatgtcgtggcagagacaaaaaaatggggtatctggtatgcgaatgaactgtcattagacggcttccgtattgatgccgccaaacatattaaattttcatttctgcgtgattgggttcaggcggtcagacaggcgacgggaaaagaaatgtttacggttgcggagtattggcagaataatgccgggaaactcgaaaactacttgaataaaacaagctttaatcaatccgtgtttgatgttccgcttcatttcaatttacaggcggcttcctcacaaggaggcggatatgatatgaggcgtttgctggacggtaccgttgtgtccaggcatccggaaaaggcggttacatttgttgaaaatcatgacacacagccgggacagtcattggaatcgacagtccaaacttggtttaaaccgcttgcatacgcctttattttgacaagagaatccggttatcctcaggtgttctatggggatatgtacgggacaaaagggacatcgccaaaggaaattccctcactgaaagataatatagagccgattttaaaagcgcgtaaggagtacgcatacgggccccagcacgattatattgaccacccggatgtgatcggatggacgagggaaggtgacagctccgccgccaaatcaggtttggccgctttaatcacggacggacccggcggatcaaagcggatgtatgccggcctgaaaaatgccggcgagacatggtatgacataacgggcaaccgttcagatactgtaaaaatcggatctgacggctggggagagtttcatgtaaacgatgggtccgtctccatttatgttcagaaa

SEQ ID NO: 4 - protein, 514 aa, Bacillus sp.
  REGION 30..514: note = Protein
MNRWKAAFSWMLSLALVFTLFYTPSSASAHHDGTNGTIMQYFEWNVPNDGQHWNRLHNNAQNLKNAGITAIWIPPAWKGTSQNDVGYGAYDLYDLGEFNQKGTVRTKYGTKAELERAIRSLKANGIQVYGDVVMNHKGGADFTERVQAVEVNPQNRNQEVSGTYQIEAWTGFNFPGRGNQHSSFKWRWYHFDGTDWDQSRQLANRIYKFRGDGKAWDWEVDTENGNYDYLMYADVDMDHPEVINELNRWGVWYANTLNLDGFRLDAVKHIKFSFMRDWLGHVRGQTGKNLFAVAEYWKNDLGALENYLSKTNWTMSAFDVPLHYNLYQASNSSGNYDMRNLLNGTLVQRHPSHAVTFVDNHDTQPGEALESFVQGWFKPLAYATILTREQGYPQVFYGDYYGIPSDGVPSYRQQIDPLLKARQQYAYGRQHDYFDHWDVIGWTREGNASHPNSGLATIMSDGPGGSKWMYVGRQKAGEVWHDMTGNRSGTVTINQDGWGHFFVNGGSVSVWVKR

SEQ ID NO: 5 - protein, 513 aa, Alicyclobacillus sp.
  REGION 28..513: note = protein
MKIRNGWKKTLTLLFALIFLLPHSAAATFAGDNGTMMQYFEWYLPNDGTLWTKMGSDASHLKSIGITGVWFPPAYKGQSQSDVGYGVYDMYDLGEFNQKGTVRTKYGTKAQLQSAITSLHNNGIQAYGDVVLNHRMGADATETISAVEVNPSNRNQVTSGAYNISAWTDFEFPGRGNTYSSFKWHSYYFDGVDWDQSRQLSGKIYQIQGTGKAWDWEVDSENGNYDYLMGADIDYDHPDVQTEVKNWGKWFVNTLNLDGVRLDAVKHIKFDYMSSWLSSVKSTTGKSNLFAVGEYWNTSLGALENYENKTNWSMSLFDVPLHMNFQAAANGGGYYDMRNLLNNTMMKNHPIQAVTFVDNHDTEPGQALQSWVSDWFKPLAYATILTRQEGYPCVFYGDYYGIPSQSVSAKSTWLDKQLSARKSYAYGTQHDYLDNQDVIGWTREGDSAHAGSGLATVMSDGPGGSKTMYVGTAHAGQVFKDITGNRTDTVTINSAGNGTFPCNGGSVSIWVKQ

SEQ ID NO: 6 - protein, 514 aa, Bacillus amyloliquefaciens
  REGION 32..514: note = protein
MIQKRKRTVSFRLVLMCTLLFVSLPITKTSAVNGTLMQYFEWYTPNDGQHWKRLQNDAEHLSDIGITAVWIPPAYKGLSQSDNGYGPYDLYDLGEFQQKGTVRTKYGTKSELQDAIGSLHSRNVQVYGDVVLNHKAGADATEDVTAVEVNPANRNQETSEEYQIKAWTDFRFPGRGNTYSDFKWHWYHFDGADWDESRKISRIFKFRGEGKAWDWEVSSENGNYDYLMYADVDYDHPDVVAETKKWGIWYANELSLDGFRIDAAKHIKFSFLRDWVQAVRQATGKEMFTVAEYWQNNAGKLENYLNKTSFNQSVFDVPLHFNLQAASSQGGGYDMRRLLDGTVVSRHPEKAVTFVENHDTQPGQSLESTVQTWFKPLAYAFILTRESGYPQVFYGDMYGTKGTSPKEIPSLKDNIEPILKARKEYAYGPQHDYIDHPDVIGWTREGDSSAAKSGLAALITDGPGGSKRMYAGLKNAGETWYDITGNRSDTVKIGSDGWGEFHVNDGSVSIYVQK

SEQ ID NO: 7 - protein, 485 aa, Bacillus sp.
HHDGTNGTIMQYFEWNVPNDGQHWNRLHNNAQNLKNAGITAIWIPPAWKGTSQNDVGYGAYDLYDLGEFNQKGTVRTKYGTKAELERAIRSLKANGIQVYGDVVMNHKGGADFTERVQAVEVNPQNRNQEVSGTYQIEAWTGFNFPGRGNQHSSFKWRWYHFDGTDWDQSRQLANRIYKFRGDGKAWDWEVDTENGNYDYLMYADVDMDHPEVINELNRWGVWYANTLNLDGFRLDAVKHIKFSFMRDWLGHVRGQTGKNLFAVAEYWKNDLGALENYLSKTNWTMSAFDVPLHYNLYQASNSSGNYDMRNLLNGTLVQRHPSHAVTFVDNHDTQPGEALESFVQGWFKPLAYATILTREQGYPQVFYGDYYGIPSDGVPSYRQQIDPLLKARQQYAYGRQHDYFDHWDVIGWTREGNASHPNSGLATIMSDGPGGSKWMYVGRQKAGEVWHDMTGNRSGTVTINQDGWGHFFVNGGSVSVWVKR

SEQ ID NO: 8 - protein, 486 aa, Alicyclobacillus sp.
TFAGDNGTMMQYFEWYLPNDGTLWTKMGSDASHLKSIGITGVWFPPAYKGQSQSDVGYGVYDMYDLGEFNQKGTVRTKYGTKAQLQSAITSLHNNGIQAYGDVVLNHRMGADATETISAVEVNPSNRNQVTSGAYNISAWTDFEFPGRGNTYSSFKWHSYYFDGVDWDQSRQLSGKIYQIQGTGKAWDWEVDSENGNYDYLMGADIDYDHPDVQTEVKNWGKWFVNTLNLDGVRLDAVKHIKFDYMSSWLSSVKSTTGKSNLFAVGEYWNTSLGALENYENKTNWSMSLFDVPLHMNFQAAANGGGYYDMRNLLNNTMMKNHPIQAVTFVDNHDTEPGQALQSWVSDWFKPLAYATILTRQEGYPCVFYGDYYGIPSQSVSAKSTWLDKQLSARKSYAYGTQHDYLDNQDVIGWTREGDSAHAGSGLATVMSDGPGGSKTMYVGTAHAGQVFKDITGNRTDTVTINSAGNGTFPCNGGSVSIWVKQ

SEQ ID NO: 9 - protein, 483 aa, Bacillus amyloliquefaciens
VNGTLMQYFEWYTPNDGQHWKRLQNDAEHLSDIGITAVWIPPAYKGLSQSDNGYGPYDLYDLGEFQQKGTVRTKYGTKSELQDAIGSLHSRNVQVYGDVVLNHKAGADATEDVTAVEVNPANRNQETSEEYQIKAWTDFRFPGRGNTYSDFKWHWYHFDGADWDESRKISRIFKFRGEGKAWDWEVSSENGNYDYLMYADVDYDHPDVVAETKKWGIWYANELSLDGFRIDAAKHIKFSFLRDWVQAVRQATGKEMFTVAEYWQNNAGKLENYLNKTSFNQSVFDVPLHFNLQAASSQGGGYDMRRLLDGTVVSRHPEKAVTFVENHDTQPGQSLESTVQTWFKPLAYAFILTRESGYPQVFYGDMYGTKGTSPKEIPSLKDNIEPILKARKEYAYGPQHDYIDHPDVIGWTREGDSSAAKSGLAALITDGPGGSKRMYAGLKNAGETWYDITGNRSDTVKIGSDGWGEFHVNDGSVSIYVQK

SEQ ID NO: 10 - protein, 399 aa, Bacillus sp.
HHDGTNGTIMQYFEWNVPNDGQHWNRLHNNAQNLKNAGITAIWIPPAWKGTSQNDVGYGAYDLYDLGEFNQKGTVRTKYGTKAELERAIRSLKANGIQVYGDVVMNHKGGADFTERVQAVEVNPQNRNQEVSGTYQIEAWTGFNFPGRGNQHSSFKWRWYHFDGTDWDQSRQLANRIYKFRGDGKAWDWEVDTENGNYDYLMYADVDMDHPEVINELNRWGVWYANTLNLDGFRLDAVKHIKFSFMRDWLGHVRGQTGKNLFAVAEYWKNDLGALENYLSKTNWTMSAFDVPLHYNLYQASNSSGNYDMRNLLNGTLVQRHPSHAVTFVDNHDTQPGEALESFVQGWFKPLAYATILTREQGYPQVFYGDYYGIPSDGVPSYRQQIDPLLKARQQYAYG

SEQ ID NO: 11 - protein, 86 aa, Alicyclobacillus sp.
TQHDYLDNQDVIGWTREGDSAHAGSGLATVMSDGPGGSKTMYVGTAHAGQVFKDITGNRTDTVTINSAGNGTFPCNGGSVSIWVKQ

SEQ ID NO: 12 - protein, 86 aa, Bacillus amyloliquefaciens
PQHDYIDHPDVIGWTREGDSSAAKSGLAALITDGPGGSKRMYAGLKNAGETWYDITGNRSDTVKIGSDGWGEFHVNDGSVSIYVQK

SEQ ID NO: 13 - protein, 485 aa, synthetic construct
  REGION 1..485: note = Fusion protein 1
HHDGTNGTIMQYFEWNVPNDGQHWNRLHNNAQNLKNAGITAIWIPPAWKGTSQNDVGYGAYDLYDLGEFNQKGTVRTKYGTKAELERAIRSLKANGIQVYGDVVMNHKGGADFTERVQAVEVNPQNRNQEVSGTYQIEAWTGFNFPGRGNQHSSFKWRWYHFDGTDWDQSRQLANRIYKFRGDGKAWDWEVDTENGNYDYLMYADVDMDHPEVINELNRWGVWYANTLNLDGFRLDAVKHIKFSFMRDWLGHVRGQTGKNLFAVAEYWKNDLGALENYLSKTNWTMSAFDVPLHYNLYQASNSSGNYDMRNLLNGTLVQRHPSHAVTFVDNHDTQPGEALESFVQGWFKPLAYATILTREQGYPQVFYGDYYGIPSDGVPSYRQQIDPLLKARQQYAYGTQHDYLDNQDVIGWTREGDSAHAGSGLATVMSDGPGGSKTMYVGTAHAGQVFKDITGNRTDTVTINSAGNGTFPCNGGSVSIWVKQ

SEQ ID NO: 14 - protein, 485 aa, synthetic construct
  REGION 1..485: note = Fusion protein 2
HHDGTNGTIMQYFEWNVPNDGQHWNRLHNNAQNLKNAGITAIWIPPAWKGTSQNDVGYGAYDLYDLGEFNQKGTVRTKYGTKAELERAIRSLKANGIQVYGDVVMNHKGGADFTERVQAVEVNPQNRNQEVSGTYQIEAWTGFNFPGRGNQHSSFKWRWYHFDGTDWDQSRQLANRIYKFRGDGKAWDWEVDTENGNYDYLMYADVDMDHPEVINELNRWGVWYANTLNLDGFRLDAVKHIKFSFMRDWLGHVRGQTGKNLFAVAEYWKNDLGALENYLSKTNWTMSAFDVPLHYNLYQASNSSGNYDMRNLLNGTLVQRHPSHAVTFVDNHDTQPGEALESFVQGWFKPLAYATILTREQGYPQVFYGDYYGIPSDGVPSYRQQIDPLLKARQQYAYGPQHDYIDHPDVIGWTREGDSSAAKSGLAALITDGPGGSKRMYAGLKNAGETWYDITGNRSDTVKIGSDGWGEFHVNDGSVSIYVQK

SEQ ID NO: 15 - protein, 483 aa, Bacillus sp.
HHDGTNGTIMQYFEWNVPNDGQHWNRLHNNAQNLKNAGITAIWIPPAWKGTSQNDVGYGAYDLYDLGEFNQKGTVRTKYGTKAELERAIRSLKANGIQVYGDVVMNHKGGADFTERVQAVEVNPQNRNQEVSGTYQIEAWTGFNFPGRGNQHSSFKWRWYHFDGTDWDQSRQLANRIYKFRGKAWDWEVDTENGNYDYLMYADVDMDHPEVINELNRWGVWYANTLNLDGFRLDAVKHIKFSFMRDWLGHVRGQTGKNLFAVAEYWKNDLGALENYLSKTNWTMSAFDVPLHYNLYQASNSSGNYDMRNLLNGTLVQRHPSHAVTFVDNHDTQPGEALESFVQGWFKPLAYATILTREQGYPQVFYGDYYGIPSDGVPSYRQQIDPLLKARQQYAYGRQHDYFDHWDVIGWTREGNASHPNSGLATIMSDGPGGSKWMYVGRQKAGEVWHDMTGNRSGTVTINQDGWGHFFVNGGSVSVWVKR

SEQ ID NO: 16 - DNA, 27 bp, synthetic construct
  misc_feature 1..27: note = Artificial sequence
  source 1..27: mol_type = other DNA
caatccaagagaaccctgatacggatg

SEQ ID NO: 17 - DNA, 23 bp, synthetic construct
  misc_feature 1..23: note = Artificial sequence
  source 1..23: mol_type = other DNA
cggaacgcctggctgacaacacg